European Patent Application EP 4 596 713 A1, published August 6, 2025. Title: DNA WITH ENHANCED RESISTANCE AGAINST EXONUCLEASES AND METHODS FOR THE PRODUCTION THEREOF. Applicant: 4basebio UK Ltd. The sequence listing filed with the application follows.

SEQUENCE LISTING (6 sequences)

SEQ ID NO: 1 - DNA, 34 bp, synthetic construct
  source 1..34: mol_type = other DNA
ataacttcgtataatgtatgctatacgaagttat

SEQ ID NO: 2 - DNA, 121 bp, synthetic construct
  source 1..121: mol_type = other DNA
cgctcgctcactgaggccgcccgggcaaagcccgggcgtcgggcgacctttggtcgcccggcctcagtgagcgagcgagcgcgcagagagggagtggccaactccatcactaggggttcct

SEQ ID NO: 3 - DNA, 200 bp, synthetic construct
  source 1..200: mol_type = other DNA
ccaatgatagtactataacttcgtataatgtatgctatacgaagttattatcagcacacaattgcccattatacgcgcgtataatggactattgtgtgctgataggtctcgccctgtctgcgtaaaattgacgcacgctcgctcactgaggccgcccgggcaaagcccgggcgtcgggcgacctttggtcgcccggcctc

SEQ ID NO: 4 - DNA, 200 bp, synthetic construct
  source 1..200: mol_type = other DNA
gaggccgggcgaccaaaggtcgcccgacgcccgggctttgcccgggcggcctcagtgagcgagcgtgcgtcaattttacgcagacagggcgagacctatcagcacacaatagtccattatacgcgcgtataatgggcaattgtgtgctgataataacttcgtatagcatacattatacgaagttatagtactatcattgg

SEQ ID NO: 5 - DNA, 200 bp, synthetic construct
  source 1..200: mol_type = other DNA
cgcgctcgctcgctcactgaggccgggcgaccaaaggtcgcccgacgcccgggctttgcccgggcggcctcagtgagcgagcgtatctctcgatccttgggctagggcgagaccataacttcgtataatgtatgctatacgaagttatagtactatcggaaagaacatgtgagcaaaaggccagcaaaaggccaggaacc

SEQ ID NO: 6 - DNA, 200 bp, synthetic construct
  source 1..200: mol_type = other DNA
ggttcctggccttttgctggccttttgctcacatgttctttccgatagtactataacttcgtatagcatacattatacgaagttatggtctcgccctagcccaaggatcgagagatacgctcgctcactgaggccgcccgggcaaagcccgggcgtcgggcgacctttggtcgcccggcctcagtgagcgagcgagcgcg